European Patent Application EP 4 628 576 A1, published October 8, 2025. Title: microRNA MOLECULES FOR USE IN METHODS FOR IMPROVING RECOMBINANT AAV PRODUCTION. Applicant: Ascend Advanced Therapies GmbH. Application EP. The sequence listing filed with the application follows.

SEQUENCE LISTING (10 sequences)

SEQ ID NO: 1 - RNA, 24 nt, Homo sapiens
  source 1..24: mol_type = other RNA
tccctgagaccctttaacctgtga

SEQ ID NO: 2 - RNA, 23 nt, Homo sapiens
  source 1..23: mol_type = other RNA
tatggcttttcattcctatgtga

SEQ ID NO: 3 - RNA, 22 nt, Homo sapiens
  source 1..22: mol_type = other RNA
ctctagagggaagcgctttctg

SEQ ID NO: 4 - RNA, 19 nt, Homo sapiens
  source 1..19: mol_type = other RNA
aggttgacatacgtttccc

SEQ ID NO: 5 - RNA, 25 nt, Homo sapiens
  source 1..25: mol_type = other RNA
ccggccaagtttgcttcatttatca

SEQ ID NO: 6 - DNA, 6197 bp, synthetic construct
  source 1..6197: mol_type = other DNA
gttgacattgattattgactagttattaatagtaatcaattacggggtcattagttcatagcccatatatggagttccgcgttacataacttacggtaaatggcccgcctggctgaccgcccaacgacccccgcccattgacgtcaataatgacgtatgttcccatagtaacgccaatagggactttccattgacgtcaatgggtggagtatttacggtaaactgcccacttggcagtacatcaagtgtatcatatgccaagtacgccccctattgacgtcaatgacggtaaatggcccgcctggcattatgcccagtacatgaccttatgggactttcctacttggcagtacatctacgtattagtcatcgctattaccatggtgatgcggttttggcagtacatcaatgggcgtggatagcggtttgactcacggggatttccaagtctccaccccattgacgtcaatgggagtttgttttggcaccaaaatcaacgggactttccaaaatgtcgtaacaactccgccccattgacgcaaatgggcggtaggcgtgtacggtgggaggtctatataagcagagctctctggctaactagagaacccactgcttactggcttatcgaaattaatacgactcactatagggagtcccaagctggctagttaagctatcaacaagtttgtacaaaaaagcaggctttaaaaccatggtgagcaagggcgaggagctgttcaccggggtggtgcccatcctggtcgagctggacggcgacgtaaacggccacaagttcagcgtgtccggcgagggcgagggcgatgccacctacggcaagctgaccctgaagttcatctgcaccaccggcaagctgcccgtgccctggcccaccctcgtgaccaccttcacctacggcgtgcagtgcttcgcccgctaccccgaccacatgaagcagcacgacttcttcaagtccgccatgcccgaaggctacgtccaggagcgcaccatcttcttcaaggacgacggcaactacaagacccgcgccgaggtgaagttcgagggcgacaccctggtgaaccgcatcgagctgaagggcatcgacttcaaggaggacggcaacatcctggggcacaagctggagtacaactacaacagccacaaggtctatatcaccgccgacaagcagaagaacggcatcaaggtgaacttcaagacccgccacaacatcgaggacggcagcgtgcagctcgccgaccactaccagcagaacacccccatcggcgacggccccgtgctgctgcccgacaaccactacctgagcacccagtccgccctgagcaaagaccccaacgagaagcgcgatcacatggtcctgctggagttcgtgaccgccgccgggatcactctcggcatggacgagctgtacaagtaagctaagcacttcgtggccgtcgatcgtttaaagggaggtagtgagtcgaccagtggatcctggaggcttgctgaaggctgtatgctgtccctgagaccctttaacctgtgagttttggccactgactgactcacaggtaagggtctcagggacaggacacaaggcctgttactagcactcacatggaacaaatggcccagatcctggaggcttgctgaaggctgtatgctgtccctgagaccctttaacctgtgagttttggccactgactgactcacaggtaagggtctcagggacaggacacaaggcctgttactagcactcacatggaacaaatggcccagatcctggaggcttgctgaaggctgtatgctgtccctgagaccctttaacctgtgagttttggccactgactgactcacaggtaagggtctcagggacaggacacaaggcctgttactagcactcacatggaacaaatggcccagatcctggaggcttgctgaaggctgtatgctgtccctgagaccctttaacctgtgagttttggccactgactgactcacaggtaagggtctcagggacaggacacaaggcctgttactagcactcacatggaacaaatggcccagatctggccgcactcgagatatctagacccagctttcttgtacaaagtggttgatctagagggcccgcggttcgctgatgggggaggctaactgaaacacggaaggagacaataccggaaggaacccgcgctatgacggcaataaaaagacagaataaaacgcacgggtgttgggtcgtttgttcataaacgcggggttcggtcccagggctggcactctgtcgataccccaccgtgaccccattggggccaatacgcccgcgtttcttccttttccccaccccaccccccaagttcgggtgaaggcccagggctcgcagccaacgtcggggcggcaggccctgccatagcatcccctatagtgagtcgtattacatggtcatagctgtttcctggcagctctggcccgtgtctcaaaatctctgatggatctgcgcagctggggctctagggggtatccccacgcgccctgtagcggcgcattaagcgcggcgggtgtggtggttacgcgcagcgtgaccgctacacttgccagcgccctagcgcccgctcctttcgctttcttcccttcctttctcgccacgttcgccggctttccccgtcaagctctaaatcgggggctccctttagggttccgatttagtgctttacggcacctcgaccccaaaaaacttgattagggtgatggttcacgtagtgggccatcgccctgatagacggtttttcgccctttgacgttggagtccacgttctttaatagtggactcttgttccaaactggaacaacactcaaccctatctcggtctattcttttgatttataagggattttgccgatttcggcctattggttaaaaaatgagctgatttaacaaaaatttaacgcgaattaattctgtggaatgtgtgtcagttagggtgtggaaagtccccaggctccccagcaggcagaagtatgcaaagcatgcatctcaattagtcagcaaccaggtgtggaaagtccccaggctccccagcaggcagaagtatgcaaagcatgcatctcaattagtcagcaaccatagtcccgcccctaactccgcccatcccgcccctaactccgcccagttccgcccattctccgccccatggctgactaattttttttatttatgcagaggccgaggccgcctctgcctctgagctattccagaagtagtgaggaggcttttttggaggcctaggcttttgcaaaaagctcccgggagcttgtatatccattttcggatctgatcagcacgtgttgacaattaatcatcggcatagtatatcggcatagtataatacgacaaggtgaggaactaaaccatggccaagcctttgtctcaagaagaatccaccctcattgaaagagcaacggctacaatcaacagcatccccatctctgaagactacagcgtcgccagcgcagctctctctagcgacggccgcatcttcactggtgtcaatgtatatcattttactgggggaccttgtgcagaactcgtggtgctgggcactgctgctgctgcggcagctggcaacctgacttgtatcgtcgcgatcggaaatgagaacaggggcatcttgagcccctgcggacggtgccgacaggtgcttctcgatctgcatcctgggatcaaagccatagtgaaggacagtgatggacagccgacggcagttgggattcgtgaattgctgccctctggttatgtgtgggagggctaagcacttcgtggccgaggagcaggactgacacgtgctacgagatttcgattccaccgccgccttctatgaaaggttgggcttcggaatcgttttccgggacgccggctggatgatcctccagcgcggggatctcatgctggagttcttcgcccaccccaacttgtttattgcagcttataatggttacaaataaagcaatagcatcacaaatttcacaaataaagcatttttttcactgcattctagttgtggtttgtccaaactcatcaatgtatcttatcatgtctgtataccgtcgctcttccgctgcttcctcgctcactgactcgctgcgctcggtcgttcggctgcggcgagcggtatcagctcactcaaaggcggtaatacggttatccacagaatcaggggataacgcaggaaagaacatgtgagcaaaaggccagcaaaaggccaggaaccgtaaaaaggccgcgttgctggcgtttttccataggctccgcccccctgacgagcatcacaaaaatcgacgctcaagtcagaggtggcgaaacccgacaggactataaagataccaggcgtttccccctggaagctccctcgtgcgctctcctgttccgaccctgccgcttaccggatacctgtccgcctttctcccttcgggaagcgtggcgctttctcatagctcacgctgtaggtatctcagttcggtgtaggtcgttcgctccaagctgggctgtgtgcacgaaccccccgttcagcccgaccgctgcgccttatccggtaactatcgtcttgagtccaacccggtaagacacgacttatcgccactggcagcagccactggtaacaggattagcagagcgaggtatgtaggcggtgctacagagttcttgaagtggtggcctaactacggctacactagaagaacagtatttggtatctgcgctctgctgaagccagttaccttcggaaaaagagttggtagctcttgatccggcaaacaaaccaccgctggtagcggtggtttttttgtttgcaagcagcagattacgcgcagaaaaaaaggatctcaagaagatcctttgatcttttctacggggtctgacgctcagtggaacgacgcgtaactcacgttaagggattttggtcatgggtggctcgacgagggttatttgccgactaccttggtgatctcgcctttcacgtagtggacaaattcttccaactgatctgcgcgcgaggccaagcgatcttcttcttgtccaagataagcctgtctagcttcaagtatgacgggctgatactgggccggcaggcgctccattgcccagtcggcagcgacatccttcggcgcgattttgccggttactgcgctgtaccaaatgcgggacaacgtaagcactacatttcgctcatcgccagcccagtcgggcggcgagttccatagcgttaaggtttcatttagcgcctcaaatagatcctgttcaggaaccggatcaaagagttcctccgccgctggacctaccaaggcaacgctatgttctcttgcttttgtcagcaagatagccagatcaatgtcgatcgtggctggctcgaagatacctgcaagaatgtcattgcgctgccattctccaaattgcagttcgcgcttagctggataacgccacggaatgatgtcgtcgtgcacaacaatggtgacttctacagcgcggagaatctcgctctctccaggggaagccgaagtttccaaaaggtcgttgatcaaagctcgccgcgttgtttcatcaagccttacggtcaccgtaaccagcaaatcaatatcactgtgtggcttcaggccgccatccactgcggagccgtacaaatgtacggccagcaacgtcggttcgagatggcgctcgatgacgccaactacctctgatagttgagtcgatacttcggcgatcaccgcttccctcataatgtttaactttgttttagggcgactgccctgctgcgtaacatcgttgctgctccataacatcaaacatcgacccacggcgtaacgcgcttgctgcttggatgcccgaggcatagactgtaccccaaaaaaacagtcataacaagccatgaaaaccgccactgcgccgttaccaccgctgcgttcggtcaaggttctggaccagttgcgtgagcgcatacgctacttgcattacagcttacgaaccgaacaggcttatgtccactgggttcgtgccttcatccgtttccacggtgtgcgtcacccggcaaccttgggtagcagcgaagtcgaggcatttctgtcctggctggtctagaattgcatgaagaatctgcttagggttaggcgttttgcgctgcttcgcgatgtacgggccagatatacgc

SEQ ID NO: 7 - RNA, 6189 nt, synthetic construct
  source 1..6189: mol_type = other RNA
gttgacattgattattgactagttattaatagtaatcaattacggggtcattagttcatagcccatatatggagttccgcgttacataacttacggtaaatggcccgcctggctgaccgcccaacgacccccgcccattgacgtcaataatgacgtatgttcccatagtaacgccaatagggactttccattgacgtcaatgggtggagtatttacggtaaactgcccacttggcagtacatcaagtgtatcatatgccaagtacgccccctattgacgtcaatgacggtaaatggcccgcctggcattatgcccagtacatgaccttatgggactttcctacttggcagtacatctacgtattagtcatcgctattaccatggtgatgcggttttggcagtacatcaatgggcgtggatagcggtttgactcacggggatttccaagtctccaccccattgacgtcaatgggagtttgttttggcaccaaaatcaacgggactttccaaaatgtcgtaacaactccgccccattgacgcaaatgggcggtaggcgtgtacggtgggaggtctatataagcagagctctctggctaactagagaacccactgcttactggcttatcgaaattaatacgactcactatagggagtcccaagctggctagttaagctatcaacaagtttgtacaaaaaagcaggctttaaaaccatggtgagcaagggcgaggagctgttcaccggggtggtgcccatcctggtcgagctggacggcgacgtaaacggccacaagttcagcgtgtccggcgagggcgagggcgatgccacctacggcaagctgaccctgaagttcatctgcaccaccggcaagctgcccgtgccctggcccaccctcgtgaccaccttcacctacggcgtgcagtgcttcgcccgctaccccgaccacatgaagcagcacgacttcttcaagtccgccatgcccgaaggctacgtccaggagcgcaccatcttcttcaaggacgacggcaactacaagacccgcgccgaggtgaagttcgagggcgacaccctggtgaaccgcatcgagctgaagggcatcgacttcaaggaggacggcaacatcctggggcacaagctggagtacaactacaacagccacaaggtctatatcaccgccgacaagcagaagaacggcatcaaggtgaacttcaagacccgccacaacatcgaggacggcagcgtgcagctcgccgaccactaccagcagaacacccccatcggcgacggccccgtgctgctgcccgacaaccactacctgagcacccagtccgccctgagcaaagaccccaacgagaagcgcgatcacatggtcctgctggagttcgtgaccgccgccgggatcactctcggcatggacgagctgtacaagtaagctaagcacttcgtggccgtcgatcgtttaaagggaggtagtgagtcgaccagtggatcctggaggcttgctgaaggctgtatgctgtatggcttttcattcctatgtgagttttggccactgactgactcacatagatgaaaagccatacaggacacaaggcctgttactagcactcacatggaacaaatggcccagatcctggaggcttgctgaaggctgtatgctgtatggcttttcattcctatgtgagttttggccactgactgactcacatagatgaaaagccatacaggacacaaggcctgttactagcactcacatggaacaaatggcccagatcctggaggcttgctgaaggctgtatgctgtatggcttttcattcctatgtgagttttggccactgactgactcacatagatgaaaagccatacaggacacaaggcctgttactagcactcacatggaacaaatggcccagatcctggaggcttgctgaaggctgtatgctgtatggcttttcattcctatgtgagttttggccactgactgactcacatagatgaaaagccatacaggacacaaggcctgttactagcactcacatggaacaaatggcccagatctggccgcactcgagatatctagacccagctttcttgtacaaagtggttgatctagagggcccgcggttcgctgatgggggaggctaactgaaacacggaaggagacaataccggaaggaacccgcgctatgacggcaataaaaagacagaataaaacgcacgggtgttgggtcgtttgttcataaacgcggggttcggtcccagggctggcactctgtcgataccccaccgtgaccccattggggccaatacgcccgcgtttcttccttttccccaccccaccccccaagttcgggtgaaggcccagggctcgcagccaacgtcggggcggcaggccctgccatagcatcccctatagtgagtcgtattacatggtcatagctgtttcctggcagctctggcccgtgtctcaaaatctctgatggatctgcgcagctggggctctagggggtatccccacgcgccctgtagcggcgcattaagcgcggcgggtgtggtggttacgcgcagcgtgaccgctacacttgccagcgccctagcgcccgctcctttcgctttcttcccttcctttctcgccacgttcgccggctttccccgtcaagctctaaatcgggggctccctttagggttccgatttagtgctttacggcacctcgaccccaaaaaacttgattagggtgatggttcacgtagtgggccatcgccctgatagacggtttttcgccctttgacgttggagtccacgttctttaatagtggactcttgttccaaactggaacaacactcaaccctatctcggtctattcttttgatttataagggattttgccgatttcggcctattggttaaaaaatgagctgatttaacaaaaatttaacgcgaattaattctgtggaatgtgtgtcagttagggtgtggaaagtccccaggctccccagcaggcagaagtatgcaaagcatgcatctcaattagtcagcaaccaggtgtggaaagtccccaggctccccagcaggcagaagtatgcaaagcatgcatctcaattagtcagcaaccatagtcccgcccctaactccgcccatcccgcccctaactccgcccagttccgcccattctccgccccatggctgactaattttttttatttatgcagaggccgaggccgcctctgcctctgagctattccagaagtagtgaggaggcttttttggaggcctaggcttttgcaaaaagctcccgggagcttgtatatccattttcggatctgatcagcacgtgttgacaattaatcatcggcatagtatatcggcatagtataatacgacaaggtgaggaactaaaccatggccaagcctttgtctcaagaagaatccaccctcattgaaagagcaacggctacaatcaacagcatccccatctctgaagactacagcgtcgccagcgcagctctctctagcgacggccgcatcttcactggtgtcaatgtatatcattttactgggggaccttgtgcagaactcgtggtgctgggcactgctgctgctgcggcagctggcaacctgacttgtatcgtcgcgatcggaaatgagaacaggggcatcttgagcccctgcggacggtgccgacaggtgcttctcgatctgcatcctgggatcaaagccatagtgaaggacagtgatggacagccgacggcagttgggattcgtgaattgctgccctctggttatgtgtgggagggctaagcacttcgtggccgaggagcaggactgacacgtgctacgagatttcgattccaccgccgccttctatgaaaggttgggcttcggaatcgttttccgggacgccggctggatgatcctccagcgcggggatctcatgctggagttcttcgcccaccccaacttgtttattgcagcttataatggttacaaataaagcaatagcatcacaaatttcacaaataaagcatttttttcactgcattctagttgtggtttgtccaaactcatcaatgtatcttatcatgtctgtataccgtcgctcttccgctgcttcctcgctcactgactcgctgcgctcggtcgttcggctgcggcgagcggtatcagctcactcaaaggcggtaatacggttatccacagaatcaggggataacgcaggaaagaacatgtgagcaaaaggccagcaaaaggccaggaaccgtaaaaaggccgcgttgctggcgtttttccataggctccgcccccctgacgagcatcacaaaaatcgacgctcaagtcagaggtggcgaaacccgacaggactataaagataccaggcgtttccccctggaagctccctcgtgcgctctcctgttccgaccctgccgcttaccggatacctgtccgcctttctcccttcgggaagcgtggcgctttctcatagctcacgctgtaggtatctcagttcggtgtaggtcgttcgctccaagctgggctgtgtgcacgaaccccccgttcagcccgaccgctgcgccttatccggtaactatcgtcttgagtccaacccggtaagacacgacttatcgccactggcagcagccactggtaacaggattagcagagcgaggtatgtaggcggtgctacagagttcttgaagtggtggcctaactacggctacactagaagaacagtatttggtatctgcgctctgctgaagccagttaccttcggaaaaagagttggtagctcttgatccggcaaacaaaccaccgctggtagcggtggtttttttgtttgcaagcagcagattacgcgcagaaaaaaaggatctcaagaagatcctttgatcttttctacggggtctgacgctcagtggaacgacgcgtaactcacgttaagggattttggtcatgggtggctcgacgagggttatttgccgactaccttggtgatctcgcctttcacgtagtggacaaattcttccaactgatctgcgcgcgaggccaagcgatcttcttcttgtccaagataagcctgtctagcttcaagtatgacgggctgatactgggccggcaggcgctccattgcccagtcggcagcgacatccttcggcgcgattttgccggttactgcgctgtaccaaatgcgggacaacgtaagcactacatttcgctcatcgccagcccagtcgggcggcgagttccatagcgttaaggtttcatttagcgcctcaaatagatcctgttcaggaaccggatcaaagagttcctccgccgctggacctaccaaggcaacgctatgttctcttgcttttgtcagcaagatagccagatcaatgtcgatcgtggctggctcgaagatacctgcaagaatgtcattgcgctgccattctccaaattgcagttcgcgcttagctggataacgccacggaatgatgtcgtcgtgcacaacaatggtgacttctacagcgcggagaatctcgctctctccaggggaagccgaagtttccaaaaggtcgttgatcaaagctcgccgcgttgtttcatcaagccttacggtcaccgtaaccagcaaatcaatatcactgtgtggcttcaggccgccatccactgcggagccgtacaaatgtacggccagcaacgtcggttcgagatggcgctcgatgacgccaactacctctgatagttgagtcgatacttcggcgatcaccgcttccctcataatgtttaactttgttttagggcgactgccctgctgcgtaacatcgttgctgctccataacatcaaacatcgacccacggcgtaacgcgcttgctgcttggatgcccgaggcatagactgtaccccaaaaaaacagtcataacaagccatgaaaaccgccactgcgccgttaccaccgctgcgttcggtcaaggttctggaccagttgcgtgagcgcatacgctacttgcattacagcttacgaaccgaacaggcttatgtccactgggttcgtgccttcatccgtttccacggtgtgcgtcacccggcaaccttgggtagcagcgaagtcgaggcatttctgtcctggctggtctagaattgcatgaagaatctgcttagggttaggcgttttgcgctgcttcgcgatgtacgggccagatatacgc

SEQ ID NO: 8 - DNA, 6181 bp, synthetic construct
  source 1..6181: mol_type = other DNA
gttgacattgattattgactagttattaatagtaatcaattacggggtcattagttcatagcccatatatggagttccgcgttacataacttacggtaaatggcccgcctggctgaccgcccaacgacccccgcccattgacgtcaataatgacgtatgttcccatagtaacgccaatagggactttccattgacgtcaatgggtggagtatttacggtaaactgcccacttggcagtacatcaagtgtatcatatgccaagtacgccccctattgacgtcaatgacggtaaatggcccgcctggcattatgcccagtacatgaccttatgggactttcctacttggcagtacatctacgtattagtcatcgctattaccatggtgatgcggttttggcagtacatcaatgggcgtggatagcggtttgactcacggggatttccaagtctccaccccattgacgtcaatgggagtttgttttggcaccaaaatcaacgggactttccaaaatgtcgtaacaactccgccccattgacgcaaatgggcggtaggcgtgtacggtgggaggtctatataagcagagctctctggctaactagagaacccactgcttactggcttatcgaaattaatacgactcactatagggagtcccaagctggctagttaagctatcaacaagtttgtacaaaaaagcaggctttaaaaccatggtgagcaagggcgaggagctgttcaccggggtggtgcccatcctggtcgagctggacggcgacgtaaacggccacaagttcagcgtgtccggcgagggcgagggcgatgccacctacggcaagctgaccctgaagttcatctgcaccaccggcaagctgcccgtgccctggcccaccctcgtgaccaccttcacctacggcgtgcagtgcttcgcccgctaccccgaccacatgaagcagcacgacttcttcaagtccgccatgcccgaaggctacgtccaggagcgcaccatcttcttcaaggacgacggcaactacaagacccgcgccgaggtgaagttcgagggcgacaccctggtgaaccgcatcgagctgaagggcatcgacttcaaggaggacggcaacatcctggggcacaagctggagtacaactacaacagccacaaggtctatatcaccgccgacaagcagaagaacggcatcaaggtgaacttcaagacccgccacaacatcgaggacggcagcgtgcagctcgccgaccactaccagcagaacacccccatcggcgacggccccgtgctgctgcccgacaaccactacctgagcacccagtccgccctgagcaaagaccccaacgagaagcgcgatcacatggtcctgctggagttcgtgaccgccgccgggatcactctcggcatggacgagctgtacaagtaagctaagcacttcgtggccgtcgatcgtttaaagggaggtagtgagtcgaccagtggatcctggaggcttgctgaaggctgtatgctgctctagagggaagcgctttctggttttggccactgactgaccagaaagcttccctctagagcaggacacaaggcctgttactagcactcacatggaacaaatggcccagatcctggaggcttgctgaaggctgtatgctgctctagagggaagcgctttctggttttggccactgactgaccagaaagcttccctctagagcaggacacaaggcctgttactagcactcacatggaacaaatggcccagatcctggaggcttgctgaaggctgtatgctgctctagagggaagcgctttctggttttggccactgactgaccagaaagcttccctctagagcaggacacaaggcctgttactagcactcacatggaacaaatggcccagatcctggaggcttgctgaaggctgtatgctgctctagagggaagcgctttctggttttggccactgactgaccagaaagcttccctctagagcaggacacaaggcctgttactagcactcacatggaacaaatggcccagatctggccgcactcgagatatctagacccagctttcttgtacaaagtggttgatctagagggcccgcggttcgctgatgggggaggctaactgaaacacggaaggagacaataccggaaggaacccgcgctatgacggcaataaaaagacagaataaaacgcacgggtgttgggtcgtttgttcataaacgcggggttcggtcccagggctggcactctgtcgataccccaccgtgaccccattggggccaatacgcccgcgtttcttccttttccccaccccaccccccaagttcgggtgaaggcccagggctcgcagccaacgtcggggcggcaggccctgccatagcatcccctatagtgagtcgtattacatggtcatagctgtttcctggcagctctggcccgtgtctcaaaatctctgatggatctgcgcagctggggctctagggggtatccccacgcgccctgtagcggcgcattaagcgcggcgggtgtggtggttacgcgcagcgtgaccgctacacttgccagcgccctagcgcccgctcctttcgctttcttcccttcctttctcgccacgttcgccggctttccccgtcaagctctaaatcgggggctccctttagggttccgatttagtgctttacggcacctcgaccccaaaaaacttgattagggtgatggttcacgtagtgggccatcgccctgatagacggtttttcgccctttgacgttggagtccacgttctttaatagtggactcttgttccaaactggaacaacactcaaccctatctcggtctattcttttgatttataagggattttgccgatttcggcctattggttaaaaaatgagctgatttaacaaaaatttaacgcgaattaattctgtggaatgtgtgtcagttagggtgtggaaagtccccaggctccccagcaggcagaagtatgcaaagcatgcatctcaattagtcagcaaccaggtgtggaaagtccccaggctccccagcaggcagaagtatgcaaagcatgcatctcaattagtcagcaaccatagtcccgcccctaactccgcccatcccgcccctaactccgcccagttccgcccattctccgccccatggctgactaattttttttatttatgcagaggccgaggccgcctctgcctctgagctattccagaagtagtgaggaggcttttttggaggcctaggcttttgcaaaaagctcccgggagcttgtatatccattttcggatctgatcagcacgtgttgacaattaatcatcggcatagtatatcggcatagtataatacgacaaggtgaggaactaaaccatggccaagcctttgtctcaagaagaatccaccctcattgaaagagcaacggctacaatcaacagcatccccatctctgaagactacagcgtcgccagcgcagctctctctagcgacggccgcatcttcactggtgtcaatgtatatcattttactgggggaccttgtgcagaactcgtggtgctgggcactgctgctgctgcggcagctggcaacctgacttgtatcgtcgcgatcggaaatgagaacaggggcatcttgagcccctgcggacggtgccgacaggtgcttctcgatctgcatcctgggatcaaagccatagtgaaggacagtgatggacagccgacggcagttgggattcgtgaattgctgccctctggttatgtgtgggagggctaagcacttcgtggccgaggagcaggactgacacgtgctacgagatttcgattccaccgccgccttctatgaaaggttgggcttcggaatcgttttccgggacgccggctggatgatcctccagcgcggggatctcatgctggagttcttcgcccaccccaacttgtttattgcagcttataatggttacaaataaagcaatagcatcacaaatttcacaaataaagcatttttttcactgcattctagttgtggtttgtccaaactcatcaatgtatcttatcatgtctgtataccgtcgctcttccgctgcttcctcgctcactgactcgctgcgctcggtcgttcggctgcggcgagcggtatcagctcactcaaaggcggtaatacggttatccacagaatcaggggataacgcaggaaagaacatgtgagcaaaaggccagcaaaaggccaggaaccgtaaaaaggccgcgttgctggcgtttttccataggctccgcccccctgacgagcatcacaaaaatcgacgctcaagtcagaggtggcgaaacccgacaggactataaagataccaggcgtttccccctggaagctccctcgtgcgctctcctgttccgaccctgccgcttaccggatacctgtccgcctttctcccttcgggaagcgtggcgctttctcatagctcacgctgtaggtatctcagttcggtgtaggtcgttcgctccaagctgggctgtgtgcacgaaccccccgttcagcccgaccgctgcgccttatccggtaactatcgtcttgagtccaacccggtaagacacgacttatcgccactggcagcagccactggtaacaggattagcagagcgaggtatgtaggcggtgctacagagttcttgaagtggtggcctaactacggctacactagaagaacagtatttggtatctgcgctctgctgaagccagttaccttcggaaaaagagttggtagctcttgatccggcaaacaaaccaccgctggtagcggtggtttttttgtttgcaagcagcagattacgcgcagaaaaaaaggatctcaagaagatcctttgatcttttctacggggtctgacgctcagtggaacgacgcgtaactcacgttaagggattttggtcatgggtggctcgacgagggttatttgccgactaccttggtgatctcgcctttcacgtagtggacaaattcttccaactgatctgcgcgcgaggccaagcgatcttcttcttgtccaagataagcctgtctagcttcaagtatgacgggctgatactgggccggcaggcgctccattgcccagtcggcagcgacatccttcggcgcgattttgccggttactgcgctgtaccaaatgcgggacaacgtaagcactacatttcgctcatcgccagcccagtcgggcggcgagttccatagcgttaaggtttcatttagcgcctcaaatagatcctgttcaggaaccggatcaaagagttcctccgccgctggacctaccaaggcaacgctatgttctcttgcttttgtcagcaagatagccagatcaatgtcgatcgtggctggctcgaagatacctgcaagaatgtcattgcgctgccattctccaaattgcagttcgcgcttagctggataacgccacggaatgatgtcgtcgtgcacaacaatggtgacttctacagcgcggagaatctcgctctctccaggggaagccgaagtttccaaaaggtcgttgatcaaagctcgccgcgttgtttcatcaagccttacggtcaccgtaaccagcaaatcaatatcactgtgtggcttcaggccgccatccactgcggagccgtacaaatgtacggccagcaacgtcggttcgagatggcgctcgatgacgccaactacctctgatagttgagtcgatacttcggcgatcaccgcttccctcataatgtttaactttgttttagggcgactgccctgctgcgtaacatcgttgctgctccataacatcaaacatcgacccacggcgtaacgcgcttgctgcttggatgcccgaggcatagactgtaccccaaaaaaacagtcataacaagccatgaaaaccgccactgcgccgttaccaccgctgcgttcggtcaaggttctggaccagttgcgtgagcgcatacgctacttgcattacagcttacgaaccgaacaggcttatgtccactgggttcgtgccttcatccgtttccacggtgtgcgtcacccggcaaccttgggtagcagcgaagtcgaggcatttctgtcctggctggtctagaattgcatgaagaatctgcttagggttaggcgttttgcgctgcttcgcgatgtacgggccagatatacgc

SEQ ID NO: 9 - DNA, 6157 bp, synthetic construct
  source 1..6157: mol_type = other DNA
gttgacattgattattgactagttattaatagtaatcaattacggggtcattagttcatagcccatatatggagttccgcgttacataacttacggtaaatggcccgcctggctgaccgcccaacgacccccgcccattgacgtcaataatgacgtatgttcccatagtaacgccaatagggactttccattgacgtcaatgggtggagtatttacggtaaactgcccacttggcagtacatcaagtgtatcatatgccaagtacgccccctattgacgtcaatgacggtaaatggcccgcctggcattatgcccagtacatgaccttatgggactttcctacttggcagtacatctacgtattagtcatcgctattaccatggtgatgcggttttggcagtacatcaatgggcgtggatagcggtttgactcacggggatttccaagtctccaccccattgacgtcaatgggagtttgttttggcaccaaaatcaacgggactttccaaaatgtcgtaacaactccgccccattgacgcaaatgggcggtaggcgtgtacggtgggaggtctatataagcagagctctctggctaactagagaacccactgcttactggcttatcgaaattaatacgactcactatagggagtcccaagctggctagttaagctatcaacaagtttgtacaaaaaagcaggctttaaaaccatggtgagcaagggcgaggagctgttcaccggggtggtgcccatcctggtcgagctggacggcgacgtaaacggccacaagttcagcgtgtccggcgagggcgagggcgatgccacctacggcaagctgaccctgaagttcatctgcaccaccggcaagctgcccgtgccctggcccaccctcgtgaccaccttcacctacggcgtgcagtgcttcgcccgctaccccgaccacatgaagcagcacgacttcttcaagtccgccatgcccgaaggctacgtccaggagcgcaccatcttcttcaaggacgacggcaactacaagacccgcgccgaggtgaagttcgagggcgacaccctggtgaaccgcatcgagctgaagggcatcgacttcaaggaggacggcaacatcctggggcacaagctggagtacaactacaacagccacaaggtctatatcaccgccgacaagcagaagaacggcatcaaggtgaacttcaagacccgccacaacatcgaggacggcagcgtgcagctcgccgaccactaccagcagaacacccccatcggcgacggccccgtgctgctgcccgacaaccactacctgagcacccagtccgccctgagcaaagaccccaacgagaagcgcgatcacatggtcctgctggagttcgtgaccgccgccgggatcactctcggcatggacgagctgtacaagtaagctaagcacttcgtggccgtcgatcgtttaaagggaggtagtgagtcgaccagtggatcctggaggcttgctgaaggctgtatgctgaggttgacatacgtttcccgttttggccactgactgacgggaaacgtgtcaacctcaggacacaaggcctgttactagcactcacatggaacaaatggcccagatcctggaggcttgctgaaggctgtatgctgaggttgacatacgtttcccgttttggccactgactgacgggaaacgtgtcaacctcaggacacaaggcctgttactagcactcacatggaacaaatggcccagatcctggaggcttgctgaaggctgtatgctgaggttgacatacgtttcccgttttggccactgactgacgggaaacgtgtcaacctcaggacacaaggcctgttactagcactcacatggaacaaatggcccagatcctggaggcttgctgaaggctgtatgctgaggttgacatacgtttcccgttttggccactgactgacgggaaacgtgtcaacctcaggacacaaggcctgttactagcactcacatggaacaaatggcccagatctggccgcactcgagatatctagacccagctttcttgtacaaagtggttgatctagagggcccgcggttcgctgatgggggaggctaactgaaacacggaaggagacaataccggaaggaacccgcgctatgacggcaataaaaagacagaataaaacgcacgggtgttgggtcgtttgttcataaacgcggggttcggtcccagggctggcactctgtcgataccccaccgtgaccccattggggccaatacgcccgcgtttcttccttttccccaccccaccccccaagttcgggtgaaggcccagggctcgcagccaacgtcggggcggcaggccctgccatagcatcccctatagtgagtcgtattacatggtcatagctgtttcctggcagctctggcccgtgtctcaaaatctctgatggatctgcgcagctggggctctagggggtatccccacgcgccctgtagcggcgcattaagcgcggcgggtgtggtggttacgcgcagcgtgaccgctacacttgccagcgccctagcgcccgctcctttcgctttcttcccttcctttctcgccacgttcgccggctttccccgtcaagctctaaatcgggggctccctttagggttccgatttagtgctttacggcacctcgaccccaaaaaacttgattagggtgatggttcacgtagtgggccatcgccctgatagacggtttttcgccctttgacgttggagtccacgttctttaatagtggactcttgttccaaactggaacaacactcaaccctatctcggtctattcttttgatttataagggattttgccgatttcggcctattggttaaaaaatgagctgatttaacaaaaatttaacgcgaattaattctgtggaatgtgtgtcagttagggtgtggaaagtccccaggctccccagcaggcagaagtatgcaaagcatgcatctcaattagtcagcaaccaggtgtggaaagtccccaggctccccagcaggcagaagtatgcaaagcatgcatctcaattagtcagcaaccatagtcccgcccctaactccgcccatcccgcccctaactccgcccagttccgcccattctccgccccatggctgactaattttttttatttatgcagaggccgaggccgcctctgcctctgagctattccagaagtagtgaggaggcttttttggaggcctaggcttttgcaaaaagctcccgggagcttgtatatccattttcggatctgatcagcacgtgttgacaattaatcatcggcatagtatatcggcatagtataatacgacaaggtgaggaactaaaccatggccaagcctttgtctcaagaagaatccaccctcattgaaagagcaacggctacaatcaacagcatccccatctctgaagactacagcgtcgccagcgcagctctctctagcgacggccgcatcttcactggtgtcaatgtatatcattttactgggggaccttgtgcagaactcgtggtgctgggcactgctgctgctgcggcagctggcaacctgacttgtatcgtcgcgatcggaaatgagaacaggggcatcttgagcccctgcggacggtgccgacaggtgcttctcgatctgcatcctgggatcaaagccatagtgaaggacagtgatggacagccgacggcagttgggattcgtgaattgctgccctctggttatgtgtgggagggctaagcacttcgtggccgaggagcaggactgacacgtgctacgagatttcgattccaccgccgccttctatgaaaggttgggcttcggaatcgttttccgggacgccggctggatgatcctccagcgcggggatctcatgctggagttcttcgcccaccccaacttgtttattgcagcttataatggttacaaataaagcaatagcatcacaaatttcacaaataaagcatttttttcactgcattctagttgtggtttgtccaaactcatcaatgtatcttatcatgtctgtataccgtcgctcttccgctgcttcctcgctcactgactcgctgcgctcggtcgttcggctgcggcgagcggtatcagctcactcaaaggcggtaatacggttatccacagaatcaggggataacgcaggaaagaacatgtgagcaaaaggccagcaaaaggccaggaaccgtaaaaaggccgcgttgctggcgtttttccataggctccgcccccctgacgagcatcacaaaaatcgacgctcaagtcagaggtggcgaaacccgacaggactataaagataccaggcgtttccccctggaagctccctcgtgcgctctcctgttccgaccctgccgcttaccggatacctgtccgcctttctcccttcgggaagcgtggcgctttctcatagctcacgctgtaggtatctcagttcggtgtaggtcgttcgctccaagctgggctgtgtgcacgaaccccccgttcagcccgaccgctgcgccttatccggtaactatcgtcttgagtccaacccggtaagacacgacttatcgccactggcagcagccactggtaacaggattagcagagcgaggtatgtaggcggtgctacagagttcttgaagtggtggcctaactacggctacactagaagaacagtatttggtatctgcgctctgctgaagccagttaccttcggaaaaagagttggtagctcttgatccggcaaacaaaccaccgctggtagcggtggtttttttgtttgcaagcagcagattacgcgcagaaaaaaaggatctcaagaagatcctttgatcttttctacggggtctgacgctcagtggaacgacgcgtaactcacgttaagggattttggtcatgggtggctcgacgagggttatttgccgactaccttggtgatctcgcctttcacgtagtggacaaattcttccaactgatctgcgcgcgaggccaagcgatcttcttcttgtccaagataagcctgtctagcttcaagtatgacgggctgatactgggccggcaggcgctccattgcccagtcggcagcgacatccttcggcgcgattttgccggttactgcgctgtaccaaatgcgggacaacgtaagcactacatttcgctcatcgccagcccagtcgggcggcgagttccatagcgttaaggtttcatttagcgcctcaaatagatcctgttcaggaaccggatcaaagagttcctccgccgctggacctaccaaggcaacgctatgttctcttgcttttgtcagcaagatagccagatcaatgtcgatcgtggctggctcgaagatacctgcaagaatgtcattgcgctgccattctccaaattgcagttcgcgcttagctggataacgccacggaatgatgtcgtcgtgcacaacaatggtgacttctacagcgcggagaatctcgctctctccaggggaagccgaagtttccaaaaggtcgttgatcaaagctcgccgcgttgtttcatcaagccttacggtcaccgtaaccagcaaatcaatatcactgtgtggcttcaggccgccatccactgcggagccgtacaaatgtacggccagcaacgtcggttcgagatggcgctcgatgacgccaactacctctgatagttgagtcgatacttcggcgatcaccgcttccctcataatgtttaactttgttttagggcgactgccctgctgcgtaacatcgttgctgctccataacatcaaacatcgacccacggcgtaacgcgcttgctgcttggatgcccgaggcatagactgtaccccaaaaaaacagtcataacaagccatgaaaaccgccactgcgccgttaccaccgctgcgttcggtcaaggttctggaccagttgcgtgagcgcatacgctacttgcattacagcttacgaaccgaacaggcttatgtccactgggttcgtgccttcatccgtttccacggtgtgcgtcacccggcaaccttgggtagcagcgaagtcgaggcatttctgtcctggctggtctagaattgcatgaagaatctgcttagggttaggcgttttgcgctgcttcgcgatgtacgggccagatatacgc

SEQ ID NO: 10 - DNA, 2843 bp, synthetic construct
  source 1..2843: mol_type = other DNA
ctaaattgtaagcgttaatattttgttaaaattcgcgttaaatttttgttaaatcagctcattttttaaccaataggccgaaatcggcaaaatcccttataaatcaaaagaatagaccgagatagggttgagtggccgctacagggcgctcccattcgccattcaggctgcgcaactgttgggaagggcgtttcggtgcgggcctcttcgctattacgccagctggcgaaagggggatgtgctgcaaggcgattaagttgggtaacgccagggttttcccagtcacgacgttgtaaaacgacggccagtgagcgcgacgtaatacgactcactatagggcgaattgaaggaaggccgtcaaggccgcatcaaataatgattttattttgactgatagtgacctgttcgttgcaacaaattgatgagcaatgcttttttataatgccaactttgtacaaaaaagcaggctttaaaggaaccaattcagtcgactggatccggtaccaaggtcgggcaggaagagggcctatttcccatgattccttcatatttgcatatacgatacaaggctgttagagagataattagaattaatttgactgtaaacacaaagatattagtacaaaatacgtgacgtagaaagtaataatttcttgggtagtttgcagttttaaaattatgttttaaaatggactatcatatgcttaccgtaacttgaaagtatttcgatttcttggctttatatatcttgtggaaaggacgaaacaccgccggccaagtttgcttcatttatcagagatgataaatgaagcaaacttggccggttttttctagacccagctttcttgtacaaagttggcattataagaaagcattgcttatcaatttgttgcaacgaacaggtcactatcagtcaaaataaaatcattatttgctgggcctcatgggccttcctttcactgcccgctttccagtcgggaaacctgtcgtgccagctgcattaacatggtcatagctgtttccttgcgtattgggcgctctccgcttcctcgctcactgactcgctgcgctcggtcgttcgggtaaagcctggggtgcctaatgagcaaaaggccagcaaaaggccaggaaccgtaaaaaggccgcgttgctggcgtttttccataggctccgcccccctgacgagcatcacaaaaatcgacgctcaagtcagaggtggcgaaacccgacaggactataaagataccaggcgtttccccctggaagctccctcgtgcgctctcctgttccgaccctgccgcttaccggatacctgtccgcctttctcccttcgggaagcgtggcgctttctcatagctcacgctgtaggtatctcagttcggtgtaggtcgttcgctccaagctgggctgtgtgcacgaaccccccgttcagcccgaccgctgcgccttatccggtaactatcgtcttgagtccaacccggtaagacacgacttatcgccactggcagcagccactggtaacaggattagcagagcgaggtatgtaggcggtgctacagagttcttgaagtggtggcctaactacggctacactagaagaacagtatttggtatctgcgctctgctgaagccagttaccttcggaaaaagagttggtagctcttgatccggcaaacaaaccaccgctggtagcggtggtttttttgtttgcaagcagcagattacgcgcagaaaaaaaggatctcaagaagatcctttgatcttttctacggggtctgacgctcagtggaacgaaaactcacgttaagggattttggtcatgagattatcaaaaaggatcttcacctagatccttttaaattaaaaatgaagttttaaatcaatctaaagtatatatgagtaaacttggtctgacagttattagaaaaattcatccagcagacgataaaacgcaatacgctggctatccggtgccgcaatgccatacagcaccagaaaacgatccgcccattcgccgcccagttcttccgcaatatcacgggtggccagcgcaatatcctgataacgatccgccacgcccagacggccgcaatcaataaagccgctaaaacggccattttccaccataatgttcggcaggcacgcatcaccatgggtcaccaccagatcttcgccatccggcatgctcgctttcagacgcgcaaacagctctgccggtgccaggccctgatgttcttcatccagatcatcctgatccaccaggcccgcttccatacgggtacgcgcacgttcaatacgatgtttcgcctgatgatcaaacggacaggtcgccgggtccagggtatgcagacgacgcatggcatccgccataatgctcactttttctgccggcgccagatggctagacagcagatcctgacccggcacttcgcccagcagcagccaatcacggcccgcttcggtcaccacatccagcaccgccgcacacggaacaccggtggtggccagccagctcagacgcgccgcttcatcctgcagctcgttcagcgcaccgctcagatcggttttcacaaacagcaccggacgaccctgcgcgctcagacgaaacaccgccgcatcagagcagccaatggtctgctgcgcccaatcatagccaaacagacgttccacccacgctgccgggctacccgcatgcaggccatcctgttcaatcatactcttcctttttcaatattattgaagcatttatcagggttattgtctcatgagcggatacatatttgaatgtatttagaaaaataaacaaataggggttccgcgcacatttccccgaaaagtgccac